European Patent Application EP 4 410 995 A1, published August 7, 2024. Title: LINEAR DNA WITH ENHANCED RESISTANCE AGAINST EXONUCLEASES AND METHODS FOR THE PRODUCTION THEREOF. Applicant: 4basebio, S.L.U. Application EP. The sequence listing filed with the application follows.

SEQUENCE LISTING (14 sequences)

SEQ ID NO: 1 - DNA, 41 bp, synthetic construct
  source 1..41: mol_type = other DNA
agggctaacatttgttggccactcaggccaacaaatgttag

SEQ ID NO: 2 - DNA, 63 bp, synthetic construct
  source 1..63: mol_type = other DNA
agggctggccactcaggccaacaaatgttagactcactaacatttgttggcctgagtggccag

SEQ ID NO: 3 - DNA, 83 bp, synthetic construct
  source 1..83: mol_type = other DNA
agggctaacatttgttggccactcaggccaacaaatgttagactcactaacatttgttggcctgagtggccaacaaatgttag

SEQ ID NO: 4 - DNA, 93 bp, synthetic construct
  source 1..93: mol_type = other DNA
agggcgagcctaacatttgttggccactcaggccaacaaatgttagactcactaacatttgttggcctgagtggccaacaaatgttaggctcg

SEQ ID NO: 5 - DNA, 103 bp, synthetic construct
  source 1..103: mol_type = other DNA
agggcgagctgagcctaacatttgttggccactcaggccaacaaatgttagactcactaacatttgttggcctgagtggccaacaaatgttaggctcagctcg

SEQ ID NO: 6 - DNA, 32 bp, synthetic construct
  source 1..32: mol_type = other DNA
agggcgagctgagcctaacatttgttggccac

SEQ ID NO: 7 - DNA, 32 bp, synthetic construct
  source 1..32: mol_type = other DNA
ctgagtggccaacaaatgttaggctcagctcg

SEQ ID NO: 8 - DNA, 39 bp, synthetic construct
  source 1..39: mol_type = other DNA
tcaggccaacaaatgttagactcactaacatttgttggc

SEQ ID NO: 9 - DNA, 20 bp, synthetic construct
  source 1..20: mol_type = other DNA
agggctaacatttgttggcc

SEQ ID NO: 10 - DNA, 16 bp, synthetic construct
  source 1..16: mol_type = other DNA
ggccaacaaatgttag

SEQ ID NO: 11 - DNA, 34 bp, synthetic construct
  source 1..34: mol_type = other DNA
ataacttcgtataatgtatgctatacgaagttat

SEQ ID NO: 12 - DNA, 40 bp, synthetic construct
  source 1..40: mol_type = other DNA
agggctaacatttgttggccactcaggccacaaatgttag

SEQ ID NO: 13 - DNA, 16 bp, synthetic construct
  source 1..16: mol_type = other DNA
ggccaacaaatgttag

SEQ ID NO: 14 - DNA, 20 bp, synthetic construct
  source 1..20: mol_type = other DNA
agggctaacatttgttggcc